European Patent Specification EP 3 476 932 B1, published November 20, 2024. Title: Novel microorganism a member of family Sporichthyaceae and uses thereof. Applicant: COSMAX, INC. The sequence listing filed with the application follows.

SEQUENCE LISTING (34 sequences)

SEQ ID NO: 1 - DNA, 1450 bp, Epidermidibacterium keratini
caggacgaacgctggcggcgtgcttaacacatgcaagtcgagcgaagctctcctcttcggaggagatgacttagcggcgaacgggtgagtaacacgtgggcaacctgcccttagctctgggataagcgatggaaacgtcgtctaataccggatacgacacggaacggcatcattaccgtgtggaaagaatttcggctaaggatgggcccgcggcctatcagcttgttggtggggtaatggcctaccaaggcttcgacgggtaaccggcctgagagggcgaccggtcacactgggactgagacacggcccagactcctacgggaggcagcagtggggaatattgcacaatgggcgaaagcctgatgcagcgacgccgcgtgagggatgacggccttcgggttgtaaacctctttcagcagggacgaagcgaaagtgacggtacctgcagaagaagcgccggccaactacgtgccagcagccgcggtaatacgtagggcgcaagcgttgtccggaattattgggcgtaaagagctcgtaggcggtttatcacgtcggctgtgaaatcccgaggcttaacctcgggcctgcagtcgatacgggttgactagagtgaagcaggggagactggaattcctggtgtagcggtgaaatgcgcagatatcaggaggaacaccggtggcgaaggcgggtctctgggctttaactgacgctgaggagcgaaagcgtgggtagcgaacaggattagataccctggtagtccacgccgtaaacggtgggcgctaggtgtggggaccattccacggtctccgtgccgcagctaacgcattaagcgccccgcctggggagtacggccgcaaggctaaaactcaaaggaattgacgggggcccgcacaagcggcggagtatgttgcttaattcgatgcaacgcgaagaaccttaccaaggcttgacatataccgaaaactcatagagatatgaggtccttttgggcggtatacaggtggtgcatggttgtcgtcagctcgtgtcgtgagatgttgggttaagtcccgcaacgagcgcaaccctcgttctatgttgccagcacgtaatggtggggactcataggagactgccggggtcaactcggaggaaggtggggatgacgtcaaatcatcatgccccttatgtcttgggctgcaaacatactacaatggccggtacaaagggctgcgataccgtaaggtggagcgaatcccaaaaagccggtctcagttcggattggggtctgcaactcgaccccatgaagtcggagtcgctagtaatcgcagatcagcaacgctgcggtgaatacgttcccgggccttgtacacaccgcccgtcaagtcatgaaagtcggtaacacccgaagccggtggcctaacctttttggagggagccgtcgaaggtgggactggcgattaggactaag

SEQ ID NO: 2 - DNA, 20 bp, Artificial Sequence
  primer for bacteria
agagtttgatcmtggctcag

SEQ ID NO: 3 - DNA, 22 bp, Artificial Sequence
  primer for bacteria
tacggytaccttgttacgactt

SEQ ID NO: 4 - DNA, 40 bp, Artificial Sequence
  GC clamp for amplification of 16s ribosomal DNA gene
cgcccggggcgcgccccgggcggggcgggggcacgggggg

SEQ ID NO: 5 - DNA, 17 bp, Artificial Sequence
  forward primer for amplification of 16s ribosomal DNA gene
cctacgggaggcagcag

SEQ ID NO: 6 - DNA, 17 bp, Artificial Sequence
  reverse primer for amplification of 16s ribosomal DNA gene
attaccgcggctgctgg

SEQ ID NO: 7 - DNA, 21 bp, Artificial Sequence
  forward primer for filaggrin
agtgcactcagggggctcaca

SEQ ID NO: 8 - DNA, 20 bp, Artificial Sequence
  reverse primer for filaggrin
ccggcttggccgtaatgtgt

SEQ ID NO: 9 - DNA, 20 bp, Artificial Sequence
  forward primer for HAS3
cttaagggttgcttgcttgc

SEQ ID NO: 10 - DNA, 20 bp, Artificial Sequence
  reverse primer for HAS3
gttcgtgggagatgaaggaa

SEQ ID NO: 11 - DNA, 33 bp, Artificial Sequence
  forward primer for claudin 1
gctctagaattctcacacgtagtctttcccgct

SEQ ID NO: 12 - DNA, 33 bp, Artificial Sequence; identical to SEQ ID NO: 11
  reverse primer for claudin 1

SEQ ID NO: 13 - DNA, 33 bp, Artificial Sequence
  forward primer for claudin 4
gctctagaattccgagcgagtcatggccaacgc

SEQ ID NO: 14 - DNA, 33 bp, Artificial Sequence; identical to SEQ ID NO: 11
  reverse primer for claudin 4

SEQ ID NO: 15 - DNA, 23 bp, Artificial Sequence
  forward primer for aSMase
actttgataactgctcctctgac

SEQ ID NO: 16 - DNA, 20 bp, Artificial Sequence
  reverse primer for aSMase
ttcgtgtccagcagagtacc

SEQ ID NO: 17 - DNA, 20 bp, Artificial Sequence
  forward primer for AQP3
agacagccccttcaggattt

SEQ ID NO: 18 - DNA, 20 bp, Artificial Sequence
  reverse primer for AQP3
tcccttgccctgaatatctg

SEQ ID NO: 19 - DNA, 20 bp, Artificial Sequence
  forward primer for TG1
ccccaagagactagcagtgg

SEQ ID NO: 20 - DNA, 20 bp, Artificial Sequence
  reverse primer for TG1
agaccaggccattcttgatg

SEQ ID NO: 21 - DNA, 22 bp, Artificial Sequence
  forward primer for CerS3
acattccacaaggcaaccattg

SEQ ID NO: 22 - DNA, 20 bp, Artificial Sequence
  reverse primer for CerS3
ctcttgattccgccgactcc

SEQ ID NO: 23 - DNA, 20 bp, Artificial Sequence
  forward primer for b-actin
ggccatctcttgctcgaagt

SEQ ID NO: 24 - DNA, 20 bp, Artificial Sequence
  reverse primer for b-actin
gacaccttcaacaccccagc

SEQ ID NO: 25 - DNA, 20 bp, Artificial Sequence
  forward primer for TNF-a
cttctccttcctgatcgtgg

SEQ ID NO: 26 - DNA, 21 bp, Artificial Sequence
  reverse primer for TNF-a
gctggttatctctcagctcca

SEQ ID NO: 27 - DNA, 24 bp, Artificial Sequence
  forward primer for IL-1a
tggctcattttccctcaaaagttg

SEQ ID NO: 28 - DNA, 25 bp, Artificial Sequence
  reverse primer for IL-1a
agaaatcgtgaaatccgaagtcaag

SEQ ID NO: 29 - DNA, 21 bp, Artificial Sequence
  forward primer for TSLP
gctatctggtgcccaggctat

SEQ ID NO: 30 - DNA, 21 bp, Artificial Sequence
  reverse primer for TSLP
cgacgccacaatccttgtaat

SEQ ID NO: 31 - DNA, 20 bp, Artificial Sequence
  forward primer for DDIT3
tgcctttctcttcggacact

SEQ ID NO: 32 - DNA, 20 bp, Artificial Sequence
  reverse primer for DDIT3
tgtgacctctgctggttctg

SEQ ID NO: 33 - DNA, 18 bp, Artificial Sequence
  forward primer for TARC
cttctctgcagcacatcc

SEQ ID NO: 34 - DNA, 19 bp, Artificial Sequence
  reverse primer for TARC
aagacctctcaaggctttg